European Patent Specification EP 3 973 970 B1, published August 28, 2024. Title: MESENCHYMAL STEM CELLS AND USES THEREFOR. Applicant: Mesoblast International Sàrl. The sequence listing filed with the application follows.

SEQUENCE LISTING (4 sequences)

SEQ ID NO: 1 - DNA, 22 bp, Artificial Sequence
  synthetic sequences and are primers for PCR derived from human        COX-1
  misc_feature (1)..(22): COX-1 forward primer
ccggatgccagtcaggatgatg

SEQ ID NO: 2 - DNA, 22 bp, Artificial Sequence
  synthetic sequences and are primers for PCR derived from human        COX-1
  misc_feature (1)..(22): COX-1 reverse primer
ctagacagccagatgctgacag

SEQ ID NO: 3 - DNA, 20 bp, Artificial Sequence
  synthetic sequences and are primers for PCR derived from human        COX-2
  misc_feature (1)..(20): COX-2 forward primer
atctaccctcctcaagtccc

SEQ ID NO: 4 - DNA, 21 bp, Artificial Sequence
  primer for PCR derived from human COX-2
  misc_feature (1)..(21): COX-2 reverse primer
taccagaagggcaggatacag